European Patent Application EP 4 144 859 A1, published March 8, 2023. Title: Tumor Detection Reagent and Kit. Applicant: Creative Biosciences (Guangzhou) Co., LTD. The sequence listing filed with the application follows.

SEQUENCE LISTING (83 sequences)

SEQ ID NO: 1 - DNA, 366 bp, Homo sapiens
  nuclear acid fragment 1 sequence
agctcggctttgccaagcgccccaggccagtaagagcggtgcagccgagccggcgccccagaagccgagaggttacacaagtctacgcagagaggcgcaccggacacggtaattaggagcaattcacacgctctcgggcgcacggaaactacttgtcaggaaattttcaacgctcctcctcgcccacttttttccactcctttcctggcgcgccccctcccctcccagaggcacgcagtggagcttttggagtttcgaatctttcggacactgcagaatgcggggctccccgggcgcgggcccggccaatcagagcgccgtctgcctcccctggccaatggcaggcgccacattgttgtccaattc

SEQ ID NO: 2 - DNA, 372 bp, Homo sapiens
  nuclear acid fragment 2 sequence
tggagccctaaggaccaacaatagagcgggcgagcggctcattgagagtctggcagcgccgggcaactgggccccggctgcgcgcagcgtccggcgcgcaccgcgaggggacccggcacggcgagagtcaggtcgcgggttccaaccacgcggcccgcagacgagcctccgacccggatttctgaagggagggttggactgcgctgcgttctgaggggtccggaagttcggacatggtgactgaaggagggtgacgtggtcagataaggggccgggggcaaagggaagcggccaagagctccagcgtcgccagtggagccgggaggcgcgtgcagcgccagcggaggaggaggatcccggagcccaaggcag

SEQ ID NO: 3 - DNA, 213 bp, Homo sapiens
  nuclear acid fragment 3 sequence
aagggtctgggagaggaggcaacgctcatagagaggaggtctgggactctcggacggagacacaaggactctgtcgcgggctctggcagggacggggaacgcgggaagcagaggagaccgcggcagaagcggggagctgggcctgcttgggccttatggggctgcggcgtgggagggactctggtgtccgtttatggccagttgcgaaggcga

SEQ ID NO: 4 - DNA, 1051 bp, Homo sapiens
  nuclear acid fragment 4 sequence
cgcggcccaaatttccctctccagcttgggttcctcaaggcggcgctttggcctagcgcgcggtgtgctcctcaccaggtctctcccctctcccaccttctttcccgtcaggtcctgtcatggagctgcgctcggagctgcccagcgtgcccggcgcggcgacggcggcggcggcaacagcgacggggccgcctgtggcgtcggtggcgtcggtggcggcagccgcggcggccgctgcatcgctaccggtgagcgtggcaggcggcttgctgcgggggccgccactgttgctgcgggcagccgagaagtacccgcggacccccaagtgcgcgcgctgtcgcaaccatggcgtggtgtcggccctcaagggccacaaacgctactgtcgctggaaggactgcctgtgcgccaagtgcacgctcatcgcggagcgccagcgtgtcatggcggcgcaggtggcgctgcgcaggcagcaggcgcaggaggagaacgaggcgcgcgagctgcagctgctctacggcactgccgaggggctggcgctggccgccgccaacggcatcatccccccgaggcccgcctacgaggtcttcggttcagtgtgcgccgccgacggcgggggacctggagcgggagcgcccgcggggaccggaggcggagcagctggcgcagggggctcaggtgagagcgcggccaggccgcaggtaggggcagcaggatcgtagctctggggcacggggcccaggggcttgtctcggttcagaaagagtagaacccccgtgtccagtcgccgcgactgctagggttcaccgctcgcccagcctcgggtatggagcgtgggtacagaaactctcctttctcccgcttctggagcatttgcactttacccctttctcctgcatcgggccgaaatgtacacgctttaatttttttactcgcctctacccaaacgcaggcaggtccctgcttctttgcttcgtcttctccccaggtggaaacctgcgcatcttcgttcgctctgcgcttctccacaggccctttccctctgctcctt

SEQ ID NO: 5 - DNA, 1200 bp, Homo sapiens
  nuclear acid fragment 5 sequence
cgacacgttttctcccctcccagaggccaagttgcagaagtttgacctgtttcctaagacgctgctgcaggcaggccgcccgggcagcccgctgccgccgccggtgaagcccttatcacccgacggcgcagactcggggcccgggacgtcgtccccagaggtgcggcccggctcaggctcggagaacggcgatggcgagtccttttctggttcgcccctagctcgggcctccaaagaggcaggtggcagctgcccaggcagcgctggccctggcggcggcggcgaggaggacagcccgggctccgctagccctctgggctctgaatccggttcagaggctgacaaagaagagggtgaggccgcgccggcgccagggctgggcggaggctcgggtccacggcagcggacgccgctggatatcttgacacgcgtgttcccaggccaccggcgaggcgtcctggagctggtgttgcagggctgcggcggcgacgtggtgcaggccatcgagcaggtgctgaaccaccaccgtgggggcctggcggccggcctgggccctgcggcgcccccagataaggccgccgtgggtgctgcagcagctgcagacgacgcgtggcccagccgcgtcgacgccgccgccgccgccgccgccgccgccggggggcctgggctgcctgcgccgctgcaggcggggcccgccgcacctccgcaccacagacccttgctggccggcgccatggcgcctggggcgctgggctcgctgagcagccgctcggccttctcgccgctgcagcccaacgccagtcacttcggtgccgacgcgggcgcctacccgctgggcgcgccgctcggcctcagccccctgcgcctggcctactccgcggcggcggcgcacagccgcggtctggccttcatggcgccctactccactgccggcttggtgcccacgctcggcttccgcccacccatggactacgcctttagcgatctcatgcgtgaccgctcggccgccgctgctgcggcggtgcacaaggagccgacctacggcggcggcctgtacgggcctatggtcaacggcgctccggagaagcagtagggcgaggggcctggcagccggccggtccccaaacaggaaccccagccctgttcccgcgggccatcgacccctcttcgcccagcgctctctctgcgccctggctgggc

SEQ ID NO: 6 - DNA, 273 bp, Homo sapiens
  nuclear acid fragment 6 sequence
gaaaacaatgccgaatcccgtcccgctcctcgagaaatagggggtgggggtggggcgctggggaaggtcgtgatttcccactcaggccgcggcgctaaggagacgcttgtccgaggtcccgtgggatctccgaccctcggggctactgggagaggagacttcctgtggtactcggaagacctatcccaccagagtggcgcggggctcacaactcccgaaggacccgcgaccgctgagcagagggaacacagtgtgtaccccagcttgggcacc

SEQ ID NO: 7 - DNA, 22 bp, Artificial Sequence
  nuclear acid fragment 1 forward primer
cgagaggttatataagtttacg

SEQ ID NO: 8 - DNA, 23 bp, Artificial Sequence
  nuclear acid fragment 1 reverse primer
aatttcctaacaaataatttccg

SEQ ID NO: 9 - DNA, 25 bp, Artificial Sequence
  nuclear acid fragment 1 probe
cgcccgaaaacgtataaattactcc

SEQ ID NO: 10 - DNA, 22 bp, Artificial Sequence
  nuclear acid fragment 2 forward primer
tttaaggattaataatagagcg

SEQ ID NO: 11 - DNA, 18 bp, Artificial Sequence
  nuclear acid fragment 2 reverse primer
gaaccgcgtaattaaaac

SEQ ID NO: 12 - DNA, 22 bp, Artificial Sequence
  nuclear acid fragment 2 probe
ctaactctcgccgtaccgaatc

SEQ ID NO: 13 - DNA, 18 bp, Artificial Sequence
  nuclear acid fragment 3 forward primer
ggacggagatataaggat

SEQ ID NO: 14 - DNA, 19 bp, Artificial Sequence
  nuclear acid fragment 3 reverse primer
ataaacgaacaccaaaatc

SEQ ID NO: 15 - DNA, 20 bp, Artificial Sequence
  nuclear acid fragment 3 probe
cgcaaccccataaaacccaa

SEQ ID NO: 16 - DNA, 18 bp, Artificial Sequence
  nuclear acid fragment 4 forward primer
gtagtcgagaagtattcg

SEQ ID NO: 17 - DNA, 19 bp, Artificial Sequence
  nuclear acid fragment 4 reverse primer
gataaacgtacacttaacg

SEQ ID NO: 18 - DNA, 21 bp, Artificial Sequence
  nuclear acid fragment 4 probe
atccttccaacgacaataacg

SEQ ID NO: 19 - DNA, 21 bp, Artificial Sequence
  nuclear acid fragment 5 forward primer
ttcgtttatttatggattacg

SEQ ID NO: 20 - DNA, 20 bp, Artificial Sequence
  nuclear acid fragment 5 reverse primer
cgtaaatcgactccttatac

SEQ ID NO: 21 - DNA, 20 bp, Artificial Sequence
  nuclear acid fragment 5 probe
aacaacgacgaccgaacgat

SEQ ID NO: 22 - DNA, 21 bp, Artificial Sequence
  nuclear acid fragment 6 forward primer
gaaaataatgtcgaatttcgt

SEQ ID NO: 23 - DNA, 18 bp, Artificial Sequence
  nuclear acid fragment 6 reverse primer
aaaatcgaaaatcccacg

SEQ ID NO: 24 - DNA, 22 bp, Artificial Sequence
  nuclear acid fragment 6 probe
ctcgaacaaacgtctccttaac

SEQ ID NO: 25 - DNA, 366 bp, Artificial Sequence
  nuclear acid fragment 1 sequence after modification
agttcggttttgttaagcgttttaggttagtaagagcggtgtagtcgagtcggcgttttagaagtcgagaggttatataagtttacgtagagaggcgtatcggatacggtaattaggagtaatttatacgttttcgggcgtacggaaattatttgttaggaaatttttaacgttttttttcgtttatttttttttattttttttttggcgcgttttttttttttttagaggtacgtagtggagtttttggagtttcgaatttttcggatattgtagaatgcggggtttttcgggcgcgggttcggttaattagagcgtcgtttgttttttttggttaatggtaggcgttatattgttgtttaattt

SEQ ID NO: 26 - DNA, 372 bp, Artificial Sequence
  nuclear acid fragment 2 sequence after modification
tggagttttaaggattaataatagagcgggcgagcggtttattgagagtttggtagcgtcgggtaattgggtttcggttgcgcgtagcgttcggcgcgtatcgcgaggggattcggtacggcgagagttaggtcgcgggttttaattacgcggttcgtagacgagttttcgattcggatttttgaagggagggttggattgcgttgcgttttgaggggttcggaagttcggatatggtgattgaaggagggtgacgtggttagataaggggtcgggggtaaagggaagcggttaagagttttagcgtcgttagtggagtcgggaggcgcgtgtagcgttagcggaggaggaggatttcggagtttaaggtag

SEQ ID NO: 27 - DNA, 213 bp, Artificial Sequence
  nuclear acid fragment 3 sequence after modification
aagggtttgggagaggaggtaacgtttatagagaggaggtttgggattttcggacggagatataaggattttgtcgcgggttttggtagggacggggaacgcgggaagtagaggagatcgcggtagaagcggggagttgggtttgtttgggttttatggggttgcggcgtgggagggattttggtgttcgtttatggttagttgcgaaggcga

SEQ ID NO: 28 - DNA, 1051 bp, Artificial Sequence
  nuclear acid fragment 4 sequence after modification
cgcggtttaaatttttttttttagtttgggttttttaaggcggcgttttggtttagcgcgcggtgtgttttttattaggtttttttttttttttattttttttttcgttaggttttgttatggagttgcgttcggagttgtttagcgtgttcggcgcggcgacggcggcggcggtaatagcgacggggtcgtttgtggcgtcggtggcgtcggtggcggtagtcgcggcggtcgttgtatcgttatcggtgagcgtggtaggcggtttgttgcgggggtcgttattgttgttgcgggtagtcgagaagtattcgcggatttttaagtgcgcgcgttgtcgtaattatggcgtggtgtcggtttttaagggttataaacgttattgtcgttggaaggattgtttgtgcgttaagtgtacgtttatcgcggagcgttagcgtgttatggcggcgtaggtggcgttgcgtaggtagtaggcgtaggaggagaacgaggcgcgcgagttgtagttgttttacggtattgtcgaggggttggcgttggtcgtcgttaacggtattattttttcgaggttcgtttacgaggttttcggtttagtgtgcgtcgtcgacggcgggggatttggagcgggagcgttcgcggggatcggaggcggagtagttggcgtagggggtttaggtgagagcgcggttaggtcgtaggtaggggtagtaggatcgtagttttggggtacggggtttaggggtttgtttcggtttagaaagagtagaattttcgtgtttagtcgtcgcgattgttagggtttatcgttcgtttagtttcgggtatggagcgtgggtatagaaatttttttttttttcgtttttggagtatttgtattttattttttttttttgtatcgggtcgaaatgtatacgttttaatttttttattcgtttttatttaaacgtaggtaggtttttgtttttttgtttcgttttttttttaggtggaaatttgcgtattttcgttcgttttgcgtttttttataggttttttttttttgtttttt

SEQ ID NO: 29 - DNA, 1200 bp, Artificial Sequence
  nuclear acid fragment 5 sequence after modification
cgatacgttttttttttttttagaggttaagttgtagaagtttgatttgttttttaagacgttgttgtaggtaggtcgttcgggtagttcgttgtcgtcgtcggtgaagtttttattattcgacggcgtagattcggggttcgggacgtcgtttttagaggtgcggttcggtttaggttcggagaacggcgatggcgagtttttttttggttcgtttttagttcgggtttttaaagaggtaggtggtagttgtttaggtagcgttggttttggcggcggcggcgaggaggatagttcgggtttcgttagttttttgggttttgaattcggtttagaggttgataaagaagagggtgaggtcgcgtcggcgttagggttgggcggaggttcgggtttacggtagcggacgtcgttggatattttgatacgcgtgtttttaggttatcggcgaggcgttttggagttggtgttgtagggttgcggcggcgacgtggtgtaggttatcgagtaggtgttgaattattatcgtgggggtttggcggtcggtttgggttttgcggcgtttttagataaggtcgtcgtgggtgttgtagtagttgtagacgacgcgtggtttagtcgcgtcgacgtcgtcgtcgtcgtcgtcgtcgtcgtcggggggtttgggttgtttgcgtcgttgtaggcggggttcgtcgtattttcgtattatagatttttgttggtcggcgttatggcgtttggggcgttgggttcgttgagtagtcgttcggttttttcgtcgttgtagtttaacgttagttatttcggtgtcgacgcgggcgtttattcgttgggcgcgtcgttcggttttagttttttgcgtttggtttatttcgcggcggcggcgtatagtcgcggtttggtttttatggcgttttattttattgtcggtttggtgtttacgttcggttttcgtttatttatggattacgtttttagcgattttatgcgtgatcgttcggtcgtcgttgttgcggcggtgtataaggagtcgatttacggcggcggtttgtacgggtttatggttaacggcgtttcggagaagtagtagggcgaggggtttggtagtcggtcggtttttaaataggaattttagttttgttttcgcgggttatcgattttttttcgtttagcgttttttttgcgttttggttgggt

SEQ ID NO: 30 - DNA, 273 bp, Artificial Sequence
  nuclear acid fragment 6 sequence after modification
gaaaataatgtcgaatttcgtttcgtttttcgagaaatagggggtgggggtggggcgttggggaaggtcgtgattttttatttaggtcgcggcgttaaggagacgtttgttcgaggtttcgtgggattttcgattttcggggttattgggagaggagattttttgtggtattcggaagatttattttattagagtggcgcggggtttataattttcgaaggattcgcgatcgttgagtagagggaatatagtgtgtattttagtttgggtatt

SEQ ID NO: 31 - DNA, 21 bp, Artificial Sequence
  CG443 forward primer
aggttcgtttacgaggttttc

SEQ ID NO: 32 - DNA, 18 bp, Artificial Sequence
  CG443 reverse primer
cctacgccaactactccg

SEQ ID NO: 33 - DNA, 19 bp, Artificial Sequence
  CG443 probe
cgaacgctcccgctccaaa

SEQ ID NO: 34 - DNA, 21 bp, Artificial Sequence
  CG447 forward primer
tgcgttaagtgtacgtttatc

SEQ ID NO: 35 - DNA, 22 bp, Artificial Sequence
  CG447 reverse primer
cgtaaaacaactacaactcgcg

SEQ ID NO: 36 - DNA, 24 bp, Artificial Sequence
  CG447 probe
ttctcctcctacgcctactaccta

SEQ ID NO: 37 - DNA, 20 bp, Artificial Sequence
  CG190 forward primer
gcgttgcgtaggtagtaggc

SEQ ID NO: 38 - DNA, 24 bp, Artificial Sequence
  CG190 reverse primer
gaacctcgaaaaaataataccgtt

SEQ ID NO: 39 - DNA, 19 bp, Artificial Sequence
  CG190 probe
aggagaacgaggcgcgcga

SEQ ID NO: 40 - DNA, 20 bp, Artificial Sequence
  CG437 forward primer
gcgttcggagttgtttagcg

SEQ ID NO: 41 - DNA, 18 bp, Artificial Sequence
  CG437 reverse primer
caccgacgccacaaacga

SEQ ID NO: 42 - DNA, 21 bp, Artificial Sequence
  CG437 probe
ctattaccgccgccgccgtcg

SEQ ID NO: 43 - DNA, 20 bp, Artificial Sequence
  CG441 forward primer
gcggtcgttgtatcgttatc

SEQ ID NO: 44 - DNA, 20 bp, Artificial Sequence
  CG441 reverse primer
gaatacttctcgactacccg

SEQ ID NO: 45 - DNA, 22 bp, Artificial Sequence
  CG441 probe
taacgacccccgcaacaaaccg

SEQ ID NO: 46 - DNA, 22 bp, Artificial Sequence
  CG446 forward primer
cgttgtatcgttatcggtgagc

SEQ ID NO: 47 - DNA, 19 bp, Artificial Sequence
  CG446 reverse primer
gcgcacttaaaaatccgcg

SEQ ID NO: 48 - DNA, 29 bp, Artificial Sequence
  CG446 probe
cttctcgactacccgcaacaacaataacg

SEQ ID NO: 49 - DNA, 20 bp, Artificial Sequence
  ACTB (internal reference gene) forward primer
ttttggattgtgaatttgtg

SEQ ID NO: 50 - DNA, 20 bp, Artificial Sequence
  ACTB (internal reference gene) reverse primer
aaacctactcctcccttaaa

SEQ ID NO: 51 - DNA, 20 bp, Artificial Sequence
  ACTB (internal reference gene) probe
ttgtgtgttgggtggtggtt

SEQ ID NO: 52 - DNA, 25 bp, Artificial Sequence
  ACTB (internal reference gene) forward primer
tggtgatggaggaggtttagtaagt

SEQ ID NO: 53 - DNA, 27 bp, Artificial Sequence
  ACTB (internal reference gene) reverse primer
aaccaataaaacctactcctcccttaa

SEQ ID NO: 54 - DNA, 19 bp, Artificial Sequence
  nuclear acid fragment 4 forward primer
gcgttcggagttgtttagc

SEQ ID NO: 55 - DNA, 17 bp, Artificial Sequence
  nuclear acid fragment 4 reverse primer
caccgacgccacaaacg

SEQ ID NO: 56 - DNA, 21 bp, Artificial Sequence
  MEIS1 forward primer
gttcgggataagatttcgggg

SEQ ID NO: 57 - DNA, 24 bp, Artificial Sequence
  MEIS1 reverse primer
taattaaaactacgcaacccgact

SEQ ID NO: 58 - DNA, 22 bp, Artificial Sequence
  NKX6-2 forward primer
agaagaagtattcgcgttcgat

SEQ ID NO: 59 - DNA, 22 bp, Artificial Sequence
  NKX6-2 reverse primer
gatcatacccaacgaataaacg

SEQ ID NO: 60 - DNA, 23 bp, Artificial Sequence
  OTX1 forward primer
gttagtagtagtagagcgggagc

SEQ ID NO: 61 - DNA, 24 bp, Artificial Sequence
  OTX1 reverse primer
gacgtaaattaaccactactttcg

SEQ ID NO: 62 - DNA, 23 bp, Artificial Sequence
  SIM2 forward primer
gtaggcgtagaggggataattcg

SEQ ID NO: 63 - DNA, 21 bp, Artificial Sequence
  SIM2 reverse primer
accccgcgctaaatctacaac

SEQ ID NO: 64 - DNA, 23 bp, Artificial Sequence
  SOX1 forward primer
taattaggatcgggttaaacggt

SEQ ID NO: 65 - DNA, 22 bp, Artificial Sequence
  SOX1 reverse primer
aaacgcttactaatctccgaat

SEQ ID NO: 66 - DNA, 26 bp, Artificial Sequence
  BARHL2 forward primer
cgttagtagtcggattataagcgaac

SEQ ID NO: 67 - DNA, 25 bp, Artificial Sequence
  BARHL2 reverse primer
aaaaattacgaaacaaacacgaccg

SEQ ID NO: 68 - DNA, 22 bp, Artificial Sequence
  ZNF154 forward primer
gttaggtttgggatagggatcg

SEQ ID NO: 69 - DNA, 20 bp, Artificial Sequence
  ZNF154 reverse primer
cgctaccatcaaactctacg

SEQ ID NO: 70 - DNA, 19 bp, Artificial Sequence
  RUNX3 forward primer
gaggtttagtacgcgttcg

SEQ ID NO: 71 - DNA, 20 bp, Artificial Sequence
  RUNX3 reverse primer
cccgcctcctaaatctatcg

SEQ ID NO: 72 - DNA, 20 bp, Artificial Sequence
  nuclear acid fragment 4 forward primer
gcgttcggagttgtttagcg

SEQ ID NO: 73 - DNA, 18 bp, Artificial Sequence
  nuclear acid fragment 4 reverse primer
caccgacgccacaaacga

SEQ ID NO: 74 - DNA, 21 bp, Artificial Sequence
  nuclear acid fragment 4 probe
ctattaccgccgccgccgtcg

SEQ ID NO: 75 - DNA, 21 bp, Artificial Sequence
  MEIS1 forward primer
gttcgggataagatttcgggg

SEQ ID NO: 76 - DNA, 24 bp, Artificial Sequence
  MEIS1 reverse primer
taattaaaactacgcaacccgact

SEQ ID NO: 77 - DNA, 22 bp, Artificial Sequence
  MEIS1 probe
cgagaggggtcgggcgagttag

SEQ ID NO: 78 - DNA, 23 bp, Artificial Sequence
  A1 forward primer
ttggattgtgaatttgtgtttgt

SEQ ID NO: 79 - DNA, 23 bp, Artificial Sequence
  A1 reverse primer
caataaaacctactcctccctta

SEQ ID NO: 80 - DNA, 22 bp, Artificial Sequence
  A2 forward primer
gatggaggaggtttagtaagtt

SEQ ID NO: 81 - DNA, 23 bp, Artificial Sequence
  A2 reverse primer
caataaaacctactcctccctta

SEQ ID NO: 82 - DNA, 25 bp, Artificial Sequence
  A3 forward primer
ggaggtttagtaagttttttggatt

SEQ ID NO: 83 - DNA, 23 bp, Artificial Sequence
  A3 reverse primer
caataaaacctactcctccctta